European Patent Specification EP 3 752 635 B1, published February 11, 2026. Title: BIOMOLECULAR PROBES AND METHODS OF DETECTING GENE AND PROTEIN EXPRESSION. Applicant: NanoString Technologies, Inc. Beechem, Joseph Kim, Dae Hoang, Margaret Gregory, Mark Piazza, Erin Zhou, Denise. The sequence listing filed with the application follows.

SEQUENCE LISTING (174 sequences)

SEQ ID NO: 1 - DNA, 34 bp, Artificial Sequence
  i7 sequence
agatcggaagagcacacgtctgaactccagtcac

SEQ ID NO: 2 - DNA, 30 bp, Artificial Sequence
  i5 sequence
acactctttccctacacgacgctcttccga

SEQ ID NO: 3 - DNA, 29 bp, Artificial Sequence
  P5 flow cell adapter
aatgatacggcgaccaccgagatctacac

SEQ ID NO: 4 - DNA, 24 bp, Artificial Sequence
  P7 flow cell adapter
atctcgtatgccgtcttctgcttg

SEQ ID NO: 5 - DNA, 78 bp, Artificial Sequence
  DSP_NGS_i501 Primer
aatgatacggcgaccaccgagatctacacgctcagatatagcctacactctttaagacgacgtcgctatggcctctcc

SEQ ID NO: 6 - DNA, 78 bp, Artificial Sequence
  DSP_NGS_i502 Primer
aatgatacggcgaccaccgagatctacacgctcagaatagaggcacactctttaagacgacgtcgctatggcctctcc

SEQ ID NO: 7 - DNA, 78 bp, Artificial Sequence
  DSP_NGS_i503 Primer
aatgatacggcgaccaccgagatctacacgctcagacctatcctacactctttaagacgacgtcgctatggcctctcc

SEQ ID NO: 8 - DNA, 78 bp, Artificial Sequence
  DSP_NGS_i504 Primer
aatgatacggcgaccaccgagatctacacgctcagaggctctgaacactctttaagacgacgtcgctatggcctctcc

SEQ ID NO: 9 - DNA, 78 bp, Artificial Sequence
  DSP_NGS_i505 Primer
aatgatacggcgaccaccgagatctacacgctcagaaggcgaagacactctttaagacgacgtcgctatggcctctcc

SEQ ID NO: 10 - DNA, 78 bp, Artificial Sequence
  DSP_NGS_i506 Primer
aatgatacggcgaccaccgagatctacacgctcagataatcttaacactctttaagacgacgtcgctatggcctctcc

SEQ ID NO: 11 - DNA, 78 bp, Artificial Sequence
  DSP_NGS_i507 Primer
aatgatacggcgaccaccgagatctacacgctcagacaggacgtacactctttaagacgacgtcgctatggcctctcc

SEQ ID NO: 12 - DNA, 78 bp, Artificial Sequence
  DSP_NGS_i508 Primer
aatgatacggcgaccaccgagatctacacgctcagagtactgacacactctttaagacgacgtcgctatggcctctcc

SEQ ID NO: 13 - DNA, 66 bp, Artificial Sequence
  NEBNext i701 Primer
caagcagaagacggcatacgagatcgagtaatgtgactggagttcagacgtgtgctcttccgatct

SEQ ID NO: 14 - DNA, 66 bp, Artificial Sequence
  NEBNext i702 Primer
caagcagaagacggcatacgagattctccggagtgactggagttcagacgtgtgctcttccgatct

SEQ ID NO: 15 - DNA, 66 bp, Artificial Sequence
  NEBNext i703 Primer
caagcagaagacggcatacgagataatgagcggtgactggagttcagacgtgtgctcttccgatct

SEQ ID NO: 16 - DNA, 66 bp, Artificial Sequence
  NEBNext i704 Primer
caagcagaagacggcatacgagatggaatctcgtgactggagttcagacgtgtgctcttccgatct

SEQ ID NO: 17 - DNA, 66 bp, Artificial Sequence
  NEBNext i705 Primer
caagcagaagacggcatacgagatttctgaatgtgactggagttcagacgtgtgctcttccgatct

SEQ ID NO: 18 - DNA, 66 bp, Artificial Sequence
  NEBNext i706 Primer
caagcagaagacggcatacgagatacgaattcgtgactggagttcagacgtgtgctcttccgatct

SEQ ID NO: 19 - DNA, 66 bp, Artificial Sequence
  NEBNext i707 Primer
caagcagaagacggcatacgagatagcttcaggtgactggagttcagacgtgtgctcttccgatct

SEQ ID NO: 20 - DNA, 66 bp, Artificial Sequence
  NEBNext i708 Primer
caagcagaagacggcatacgagatgcgcattagtgactggagttcagacgtgtgctcttccgatct

SEQ ID NO: 21 - DNA, 66 bp, Artificial Sequence
  NEBNext i709 Primer
caagcagaagacggcatacgagatcatagccggtgactggagttcagacgtgtgctcttccgatct

SEQ ID NO: 22 - DNA, 66 bp, Artificial Sequence
  NEBNext i710 Primer
caagcagaagacggcatacgagatttcgcggagtgactggagttcagacgtgtgctcttccgatct

SEQ ID NO: 23 - DNA, 66 bp, Artificial Sequence
  NEBNext i711 Primer
caagcagaagacggcatacgagatgcgcgagagtgactggagttcagacgtgtgctcttccgatct

SEQ ID NO: 24 - DNA, 66 bp, Artificial Sequence
  NEBNext i712 Primer
caagcagaagacggcatacgagatctatcgctgtgactggagttcagacgtgtgctcttccgatct

SEQ ID NO: 25 - DNA, 34 bp, Artificial Sequence
  Spike-in primer
acactctttaagacgacgtcgctatggcctctcc

SEQ ID NO: 26 - DNA, 34 bp, Artificial Sequence
  Amplification primer binding site
gtgactggagttcagacgtgtgctcttccgatct

SEQ ID NO: 27 - DNA, 83 bp, Artificial Sequence
  P01_PriExtUMI15_tpt
  misc_feature (35)..(49): n is a, c, g, or t
gtgactggagttcagacgtgtgctcttccgatctnnnnnnnnnnnnnnnttgaagcacaccgtttttctttcttctttcacgg

SEQ ID NO: 28 - DNA, 83 bp, Artificial Sequence
  P03_PriExtUMI15_tpt
  misc_feature (35)..(49): n is a, c, g, or t
gtgactggagttcagacgtgtgctcttccgatctnnnnnnnnnnnnnnnacccacaggttatacgggattatccggttatcca

SEQ ID NO: 29 - DNA, 83 bp, Artificial Sequence
  P04_PriExtUMI15_tpt
  misc_feature (35)..(49): n is a, c, g, or t
gtgactggagttcagacgtgtgctcttccgatctnnnnnnnnnnnnnnncgacaccgagttcgaccgttatgttggtaggatc

SEQ ID NO: 30 - DNA, 83 bp, Artificial Sequence
  P05_PriExtUMI15_tpt
  misc_feature (35)..(49): n is a, c, g, or t
gtgactggagttcagacgtgtgctcttccgatctnnnnnnnnnnnnnnncggtgtgtaagcgtaacgatgttggtgtcgctct

SEQ ID NO: 31 - DNA, 83 bp, Artificial Sequence
  P06_PriExtUMI15_tpt
  misc_feature (35)..(49): n is a, c, g, or t
gtgactggagttcagacgtgtgctcttccgatctnnnnnnnnnnnnnnncagacactgcgacaactcacgatcatgacacaga

SEQ ID NO: 32 - DNA, 83 bp, Artificial Sequence
  P07_PriExtUMI15_tpt
  misc_feature (35)..(49): n is a, c, g, or t
gtgactggagttcagacgtgtgctcttccgatctnnnnnnnnnnnnnnnatattctgtactcagtgcctatccacctaatagg

SEQ ID NO: 33 - DNA, 83 bp, Artificial Sequence
  P09_PriExtUMI15_tpt
  misc_feature (35)..(49): n is a, c, g, or t
gtgactggagttcagacgtgtgctcttccgatctnnnnnnnnnnnnnnnttcagttataatgtgtccagcagaagcaggaatt

SEQ ID NO: 34 - DNA, 83 bp, Artificial Sequence
  P11_PriExtUMI15_tpt
  misc_feature (35)..(49): n is a, c, g, or t
gtgactggagttcagacgtgtgctcttccgatctnnnnnnnnnnnnnnngtcctttgttgggcggaccgtaatgaggaatttg

SEQ ID NO: 35 - DNA, 83 bp, Artificial Sequence
  P13_PriExtUMI15_tpt
  misc_feature (35)..(49): n is a, c, g, or t
gtgactggagttcagacgtgtgctcttccgatctnnnnnnnnnnnnnnngatgagacttctacatgtccgatgtttttgtgct

SEQ ID NO: 36 - DNA, 83 bp, Artificial Sequence
  P15_PriExtUMI15_tpt
  misc_feature (35)..(49): n is a, c, g, or t
gtgactggagttcagacgtgtgctcttccgatctnnnnnnnnnnnnnnnactcacacatagtactgacacgtaagataggatg

SEQ ID NO: 37 - DNA, 83 bp, Artificial Sequence
  P16_PriExtUMI15_tpt
  misc_feature (35)..(49): n is a, c, g, or t
gtgactggagttcagacgtgtgctcttccgatctnnnnnnnnnnnnnnnttaccctatctcgtctatgtacgtcaggctgaat

SEQ ID NO: 38 - DNA, 83 bp, Artificial Sequence
  P17_PriExtUMI15_tpt
  misc_feature (35)..(49): n is a, c, g, or t
gtgactggagttcagacgtgtgctcttccgatctnnnnnnnnnnnnnnnatcaacgtagggtaaggtcatatttttaccttac

SEQ ID NO: 39 - DNA, 83 bp, Artificial Sequence
  P18_PriExtUMI15_tpt
  misc_feature (35)..(49): n is a, c, g, or t
gtgactggagttcagacgtgtgctcttccgatctnnnnnnnnnnnnnnnttccctctttctccgcttatggatgaaaggacag

SEQ ID NO: 40 - DNA, 83 bp, Artificial Sequence
  P19_PriExtUMI15_tpt
  misc_feature (35)..(49): n is a, c, g, or t
gtgactggagttcagacgtgtgctcttccgatctnnnnnnnnnnnnnnncctgcacagtgagtttctttcactctaactctct

SEQ ID NO: 41 - DNA, 83 bp, Artificial Sequence
  P20_PriExtUMI15_tpt
  misc_feature (35)..(49): n is a, c, g, or t
gtgactggagttcagacgtgtgctcttccgatctnnnnnnnnnnnnnnntgtcgctctagtgtgacttttccacctcgcatct

SEQ ID NO: 42 - DNA, 83 bp, Artificial Sequence
  P21_PriExtUMI15_tpt
  misc_feature (35)..(49): n is a, c, g, or t
gtgactggagttcagacgtgtgctcttccgatctnnnnnnnnnnnnnnnatatctttctcgggtaaagattaggcgtccgata

SEQ ID NO: 43 - DNA, 83 bp, Artificial Sequence
  P23_PriExtUMI15_tpt
  misc_feature (35)..(49): n is a, c, g, or t
gtgactggagttcagacgtgtgctcttccgatctnnnnnnnnnnnnnnncgattagccgtagacgcaactcattgccgaagat

SEQ ID NO: 44 - DNA, 83 bp, Artificial Sequence
  P24_PriExtUMI15_tpt
  misc_feature (35)..(49): n is a, c, g, or t
gtgactggagttcagacgtgtgctcttccgatctnnnnnnnnnnnnnnntgtgagcatttcagtacgagtgatgcagataaac

SEQ ID NO: 45 - DNA, 83 bp, Artificial Sequence
  P25_PriExtUMI15_tpt
  misc_feature (35)..(49): n is a, c, g, or t
gtgactggagttcagacgtgtgctcttccgatctnnnnnnnnnnnnnnntatagttaccaagtactatgggttggtggaagcc

SEQ ID NO: 46 - DNA, 83 bp, Artificial Sequence
  P26_PriExtUMI15_tpt
  misc_feature (35)..(49): n is a, c, g, or t
gtgactggagttcagacgtgtgctcttccgatctnnnnnnnnnnnnnnnccaattatactgtctgttatgttctcggataagc

SEQ ID NO: 47 - DNA, 83 bp, Artificial Sequence
  P27_PriExtUMI15_tpt
  misc_feature (35)..(49): n is a, c, g, or t
gtgactggagttcagacgtgtgctcttccgatctnnnnnnnnnnnnnnntcaggtgcttgtaggctcatgataggggtaatgc

SEQ ID NO: 48 - DNA, 83 bp, Artificial Sequence
  P28_PriExtUMI15_tpt
  misc_feature (35)..(49): n is a, c, g, or t
gtgactggagttcagacgtgtgctcttccgatctnnnnnnnnnnnnnnnctctgctgtaatctcagctccacttgtttctaag

SEQ ID NO: 49 - DNA, 83 bp, Artificial Sequence
  P29_PriExtUMI15_tpt
  misc_feature (35)..(49): n is a, c, g, or t
gtgactggagttcagacgtgtgctcttccgatctnnnnnnnnnnnnnnngtgcatattgcagctgagccagctcaatttgaag

SEQ ID NO: 50 - DNA, 83 bp, Artificial Sequence
  P30_PriExtUMI15_tpt
  misc_feature (35)..(49): n is a, c, g, or t
gtgactggagttcagacgtgtgctcttccgatctnnnnnnnnnnnnnnnccgttgatttacgcaacagcggcttatatagctc

SEQ ID NO: 51 - DNA, 83 bp, Artificial Sequence
  P31_PriExtUMI15_tpt
  misc_feature (35)..(49): n is a, c, g, or t
gtgactggagttcagacgtgtgctcttccgatctnnnnnnnnnnnnnnncatcatcgacagttcgcagccctataacatgata

SEQ ID NO: 52 - DNA, 83 bp, Artificial Sequence
  P32_PriExtUMI15_tpt
  misc_feature (35)..(49): n is a, c, g, or t
gtgactggagttcagacgtgtgctcttccgatctnnnnnnnnnnnnnnnatcgcaggatggtacagcatcatacatgatgagc

SEQ ID NO: 53 - DNA, 83 bp, Artificial Sequence; identical to SEQ ID NO: 52
  P33_PriExtUMI15_tpt
  misc_feature (35)..(49): n is a, c, g, or t

SEQ ID NO: 54 - DNA, 83 bp, Artificial Sequence
  P34_PriExtUMI15_tpt
  misc_feature (35)..(49): n is a, c, g, or t
gtgactggagttcagacgtgtgctcttccgatctnnnnnnnnnnnnnnnatggcggtttcgggtcctgcactattcctaataa

SEQ ID NO: 55 - DNA, 83 bp, Artificial Sequence
  P35_PriExtUMI15_tpt
  misc_feature (35)..(49): n is a, c, g, or t
gtgactggagttcagacgtgtgctcttccgatctnnnnnnnnnnnnnnnccagtacgggtactaataagtgtcatatctattg

SEQ ID NO: 56 - DNA, 83 bp, Artificial Sequence
  P36_PriExtUMI15_tpt
  misc_feature (35)..(49): n is a, c, g, or t
gtgactggagttcagacgtgtgctcttccgatctnnnnnnnnnnnnnnntgttggagaggttagaggtgaggaggcgaagata

SEQ ID NO: 57 - DNA, 66 bp, Artificial Sequence
  Reverse primer
caagcagaagacggcatacgagatgtcggtaagtgactggagttcagacgtgtgctcttccgatct

SEQ ID NO: 58 - DNA, 66 bp, Artificial Sequence
  Reverse primer
caagcagaagacggcatacgagataggtcactgtgactggagttcagacgtgtgctcttccgatct

SEQ ID NO: 59 - DNA, 66 bp, Artificial Sequence
  Reverse primer
caagcagaagacggcatacgagatgaatccgagtgactggagttcagacgtgtgctcttccgatct

SEQ ID NO: 60 - DNA, 66 bp, Artificial Sequence
  Reverse primer
caagcagaagacggcatacgagatgtaccttggtgactggagttcagacgtgtgctcttccgatct

SEQ ID NO: 61 - DNA, 66 bp, Artificial Sequence
  Reverse primer
caagcagaagacggcatacgagatcatgaggagtgactggagttcagacgtgtgctcttccgatct

SEQ ID NO: 62 - DNA, 66 bp, Artificial Sequence
  Reverse primer
caagcagaagacggcatacgagattgactgacgtgactggagttcagacgtgtgctcttccgatct

SEQ ID NO: 63 - DNA, 66 bp, Artificial Sequence
  Reverse primer
caagcagaagacggcatacgagatcgtattcggtgactggagttcagacgtgtgctcttccgatct

SEQ ID NO: 64 - DNA, 66 bp, Artificial Sequence
  Reverse primer
caagcagaagacggcatacgagatctcctagagtgactggagttcagacgtgtgctcttccgatct

SEQ ID NO: 65 - DNA, 66 bp, Artificial Sequence
  Reverse primer
caagcagaagacggcatacgagattagttgcggtgactggagttcagacgtgtgctcttccgatct

SEQ ID NO: 66 - DNA, 66 bp, Artificial Sequence
  Reverse primer
caagcagaagacggcatacgagatgagatacggtgactggagttcagacgtgtgctcttccgatct

SEQ ID NO: 67 - DNA, 66 bp, Artificial Sequence
  Reverse primer
caagcagaagacggcatacgagataggtgtacgtgactggagttcagacgtgtgctcttccgatct

SEQ ID NO: 68 - DNA, 66 bp, Artificial Sequence
  Reverse primer
caagcagaagacggcatacgagattaatgccggtgactggagttcagacgtgtgctcttccgatct

SEQ ID NO: 69 - DNA, 66 bp, Artificial Sequence
  Reverse primer
caagcagaagacggcatacgagattcagacgagtgactggagttcagacgtgtgctcttccgatct

SEQ ID NO: 70 - DNA, 66 bp, Artificial Sequence
  Reverse primer
caagcagaagacggcatacgagatgataggctgtgactggagttcagacgtgtgctcttccgatct

SEQ ID NO: 71 - DNA, 66 bp, Artificial Sequence
  Reverse primer
caagcagaagacggcatacgagattggtacaggtgactggagttcagacgtgtgctcttccgatct

SEQ ID NO: 72 - DNA, 66 bp, Artificial Sequence
  Reverse primer
caagcagaagacggcatacgagatcaaggtctgtgactggagttcagacgtgtgctcttccgatct

SEQ ID NO: 73 - DNA, 66 bp, Artificial Sequence
  Reverse primer
caagcagaagacggcatacgagatgctatcctgtgactggagttcagacgtgtgctcttccgatct

SEQ ID NO: 74 - DNA, 66 bp, Artificial Sequence
  Reverse primer
caagcagaagacggcatacgagatatggaagggtgactggagttcagacgtgtgctcttccgatct

SEQ ID NO: 75 - DNA, 66 bp, Artificial Sequence
  Reverse primer
caagcagaagacggcatacgagattcaaggacgtgactggagttcagacgtgtgctcttccgatct

SEQ ID NO: 76 - DNA, 66 bp, Artificial Sequence
  Reverse primer
caagcagaagacggcatacgagatgttacgcagtgactggagttcagacgtgtgctcttccgatct

SEQ ID NO: 77 - DNA, 66 bp, Artificial Sequence
  Reverse primer
caagcagaagacggcatacgagatagtctgtggtgactggagttcagacgtgtgctcttccgatct

SEQ ID NO: 78 - DNA, 66 bp, Artificial Sequence
  Reverse primer
caagcagaagacggcatacgagatgcacgtaagtgactggagttcagacgtgtgctcttccgatct

SEQ ID NO: 79 - DNA, 66 bp, Artificial Sequence
  Reverse primer
caagcagaagacggcatacgagataaccttgggtgactggagttcagacgtgtgctcttccgatct

SEQ ID NO: 80 - DNA, 66 bp, Artificial Sequence
  Reverse primer
caagcagaagacggcatacgagatattgcgtggtgactggagttcagacgtgtgctcttccgatct

SEQ ID NO: 81 - DNA, 66 bp, Artificial Sequence
  Reverse primer
caagcagaagacggcatacgagatacctggaagtgactggagttcagacgtgtgctcttccgatct

SEQ ID NO: 82 - DNA, 66 bp, Artificial Sequence
  Reverse primer
caagcagaagacggcatacgagatggagatgagtgactggagttcagacgtgtgctcttccgatct

SEQ ID NO: 83 - DNA, 66 bp, Artificial Sequence
  Reverse primer
caagcagaagacggcatacgagatgtactctcgtgactggagttcagacgtgtgctcttccgatct

SEQ ID NO: 84 - DNA, 66 bp, Artificial Sequence
  Reverse primer
caagcagaagacggcatacgagatgtaacgacgtgactggagttcagacgtgtgctcttccgatct

SEQ ID NO: 85 - DNA, 66 bp, Artificial Sequence
  Reverse primer
caagcagaagacggcatacgagatattcctccgtgactggagttcagacgtgtgctcttccgatct

SEQ ID NO: 86 - DNA, 66 bp, Artificial Sequence
  Reverse primer
caagcagaagacggcatacgagatgtgttcctgtgactggagttcagacgtgtgctcttccgatct

SEQ ID NO: 87 - DNA, 66 bp, Artificial Sequence
  Reverse primer
caagcagaagacggcatacgagataagcactggtgactggagttcagacgtgtgctcttccgatct

SEQ ID NO: 88 - DNA, 66 bp, Artificial Sequence
  Reverse primer
caagcagaagacggcatacgagatctagcaaggtgactggagttcagacgtgtgctcttccgatct

SEQ ID NO: 89 - DNA, 66 bp, Artificial Sequence
  Reverse primer
caagcagaagacggcatacgagattgcttccagtgactggagttcagacgtgtgctcttccgatct

SEQ ID NO: 90 - DNA, 66 bp, Artificial Sequence
  Reverse primer
caagcagaagacggcatacgagatgcttagctgtgactggagttcagacgtgtgctcttccgatct

SEQ ID NO: 91 - DNA, 66 bp, Artificial Sequence
  Reverse primer
caagcagaagacggcatacgagataaccgttcgtgactggagttcagacgtgtgctcttccgatct

SEQ ID NO: 92 - DNA, 66 bp, Artificial Sequence
  Reverse primer
caagcagaagacggcatacgagatgacattccgtgactggagttcagacgtgtgctcttccgatct

SEQ ID NO: 93 - DNA, 66 bp, Artificial Sequence
  Reverse primer
caagcagaagacggcatacgagatagaccgtagtgactggagttcagacgtgtgctcttccgatct

SEQ ID NO: 94 - DNA, 66 bp, Artificial Sequence
  Reverse primer
caagcagaagacggcatacgagatgatactgggtgactggagttcagacgtgtgctcttccgatct

SEQ ID NO: 95 - DNA, 66 bp, Artificial Sequence
  Reverse primer
caagcagaagacggcatacgagattgcgtagagtgactggagttcagacgtgtgctcttccgatct

SEQ ID NO: 96 - DNA, 66 bp, Artificial Sequence
  Reverse primer
caagcagaagacggcatacgagattcggttacgtgactggagttcagacgtgtgctcttccgatct

SEQ ID NO: 97 - DNA, 66 bp, Artificial Sequence
  Reverse primer
caagcagaagacggcatacgagatatgacgtcgtgactggagttcagacgtgtgctcttccgatct

SEQ ID NO: 98 - DNA, 66 bp, Artificial Sequence
  Reverse primer
caagcagaagacggcatacgagatgctgtaaggtgactggagttcagacgtgtgctcttccgatct

SEQ ID NO: 99 - DNA, 66 bp, Artificial Sequence
  Reverse primer
caagcagaagacggcatacgagatgcaatggagtgactggagttcagacgtgtgctcttccgatct

SEQ ID NO: 100 - DNA, 66 bp, Artificial Sequence
  Reverse primer
caagcagaagacggcatacgagatatctcgctgtgactggagttcagacgtgtgctcttccgatct

SEQ ID NO: 101 - DNA, 66 bp, Artificial Sequence
  Reverse primer
caagcagaagacggcatacgagatggctattggtgactggagttcagacgtgtgctcttccgatct

SEQ ID NO: 102 - DNA, 66 bp, Artificial Sequence
  Reverse primer
caagcagaagacggcatacgagatggtgtcttgtgactggagttcagacgtgtgctcttccgatct

SEQ ID NO: 103 - DNA, 66 bp, Artificial Sequence
  Reverse primer
caagcagaagacggcatacgagattcaactgggtgactggagttcagacgtgtgctcttccgatct

SEQ ID NO: 104 - DNA, 66 bp, Artificial Sequence
  Reverse primer
caagcagaagacggcatacgagatcttcaccagtgactggagttcagacgtgtgctcttccgatct

SEQ ID NO: 105 - DNA, 66 bp, Artificial Sequence
  Reverse primer
caagcagaagacggcatacgagatacggtcttgtgactggagttcagacgtgtgctcttccgatct

SEQ ID NO: 106 - DNA, 66 bp, Artificial Sequence
  Reverse primer
caagcagaagacggcatacgagattctcgcaagtgactggagttcagacgtgtgctcttccgatct

SEQ ID NO: 107 - DNA, 66 bp, Artificial Sequence
  Reverse primer
caagcagaagacggcatacgagatggaattgcgtgactggagttcagacgtgtgctcttccgatct

SEQ ID NO: 108 - DNA, 66 bp, Artificial Sequence
  Reverse primer
caagcagaagacggcatacgagatacggattcgtgactggagttcagacgtgtgctcttccgatct

SEQ ID NO: 109 - DNA, 66 bp, Artificial Sequence
  Reverse primer
caagcagaagacggcatacgagatttaagcgggtgactggagttcagacgtgtgctcttccgatct

SEQ ID NO: 110 - DNA, 66 bp, Artificial Sequence
  Reverse primer
caagcagaagacggcatacgagattgcaggtagtgactggagttcagacgtgtgctcttccgatct

SEQ ID NO: 111 - DNA, 66 bp, Artificial Sequence
  Reverse primer
caagcagaagacggcatacgagatcaatcgacgtgactggagttcagacgtgtgctcttccgatct

SEQ ID NO: 112 - DNA, 66 bp, Artificial Sequence
  Reverse primer
caagcagaagacggcatacgagatgtgccatagtgactggagttcagacgtgtgctcttccgatct

SEQ ID NO: 113 - DNA, 66 bp, Artificial Sequence
  Reverse primer
caagcagaagacggcatacgagattgttcgaggtgactggagttcagacgtgtgctcttccgatct

SEQ ID NO: 114 - DNA, 66 bp, Artificial Sequence
  Reverse primer
caagcagaagacggcatacgagattggagttggtgactggagttcagacgtgtgctcttccgatct

SEQ ID NO: 115 - DNA, 66 bp, Artificial Sequence
  Reverse primer
caagcagaagacggcatacgagatacgatgacgtgactggagttcagacgtgtgctcttccgatct

SEQ ID NO: 116 - DNA, 66 bp, Artificial Sequence
  Reverse primer
caagcagaagacggcatacgagattgatgtccgtgactggagttcagacgtgtgctcttccgatct

SEQ ID NO: 117 - DNA, 66 bp, Artificial Sequence
  Reverse primer
caagcagaagacggcatacgagattgaacctggtgactggagttcagacgtgtgctcttccgatct

SEQ ID NO: 118 - DNA, 66 bp, Artificial Sequence
  Reverse primer
caagcagaagacggcatacgagatcttcgttcgtgactggagttcagacgtgtgctcttccgatct

SEQ ID NO: 119 - DNA, 66 bp, Artificial Sequence
  Reverse primer
caagcagaagacggcatacgagatcttctgaggtgactggagttcagacgtgtgctcttccgatct

SEQ ID NO: 120 - DNA, 66 bp, Artificial Sequence
  Reverse primer
caagcagaagacggcatacgagattgctcatggtgactggagttcagacgtgtgctcttccgatct

SEQ ID NO: 121 - DNA, 66 bp, Artificial Sequence
  Reverse primer
caagcagaagacggcatacgagatagttcgtcgtgactggagttcagacgtgtgctcttccgatct

SEQ ID NO: 122 - DNA, 66 bp, Artificial Sequence
  Reverse primer
caagcagaagacggcatacgagattagcgtctgtgactggagttcagacgtgtgctcttccgatct

SEQ ID NO: 123 - DNA, 66 bp, Artificial Sequence
  Reverse primer
caagcagaagacggcatacgagatggcgttatgtgactggagttcagacgtgtgctcttccgatct

SEQ ID NO: 124 - DNA, 66 bp, Artificial Sequence
  Reverse primer
caagcagaagacggcatacgagatggtgattcgtgactggagttcagacgtgtgctcttccgatct

SEQ ID NO: 125 - DNA, 66 bp, Artificial Sequence
  Reverse primer
caagcagaagacggcatacgagataacttgccgtgactggagttcagacgtgtgctcttccgatct

SEQ ID NO: 126 - DNA, 66 bp, Artificial Sequence
  Reverse primer
caagcagaagacggcatacgagatgcaagatcgtgactggagttcagacgtgtgctcttccgatct

SEQ ID NO: 127 - DNA, 66 bp, Artificial Sequence
  Reverse primer
caagcagaagacggcatacgagattcgcattggtgactggagttcagacgtgtgctcttccgatct

SEQ ID NO: 128 - DNA, 66 bp, Artificial Sequence
  Reverse primer
caagcagaagacggcatacgagattgtacaccgtgactggagttcagacgtgtgctcttccgatct

SEQ ID NO: 129 - DNA, 66 bp, Artificial Sequence
  Reverse primer
caagcagaagacggcatacgagatagctcctagtgactggagttcagacgtgtgctcttccgatct

SEQ ID NO: 130 - DNA, 66 bp, Artificial Sequence
  Reverse primer
caagcagaagacggcatacgagatgcaattcggtgactggagttcagacgtgtgctcttccgatct

SEQ ID NO: 131 - DNA, 66 bp, Artificial Sequence
  Reverse primer
caagcagaagacggcatacgagatcttaggacgtgactggagttcagacgtgtgctcttccgatct

SEQ ID NO: 132 - DNA, 66 bp, Artificial Sequence
  Reverse primer
caagcagaagacggcatacgagatgtcctaaggtgactggagttcagacgtgtgctcttccgatct

SEQ ID NO: 133 - DNA, 66 bp, Artificial Sequence
  Reverse primer
caagcagaagacggcatacgagataacgtggagtgactggagttcagacgtgtgctcttccgatct

SEQ ID NO: 134 - DNA, 66 bp, Artificial Sequence
  Reverse primer
caagcagaagacggcatacgagatctgtgttggtgactggagttcagacgtgtgctcttccgatct

SEQ ID NO: 135 - DNA, 66 bp, Artificial Sequence
  Reverse primer
caagcagaagacggcatacgagatgttaaggcgtgactggagttcagacgtgtgctcttccgatct

SEQ ID NO: 136 - DNA, 66 bp, Artificial Sequence
  Reverse primer
caagcagaagacggcatacgagatcaccttacgtgactggagttcagacgtgtgctcttccgatct

SEQ ID NO: 137 - DNA, 66 bp, Artificial Sequence
  Reverse primer
caagcagaagacggcatacgagattggtagctgtgactggagttcagacgtgtgctcttccgatct

SEQ ID NO: 138 - DNA, 66 bp, Artificial Sequence
  Reverse primer
caagcagaagacggcatacgagatcagtgaaggtgactggagttcagacgtgtgctcttccgatct

SEQ ID NO: 139 - DNA, 66 bp, Artificial Sequence
  Reverse primer
caagcagaagacggcatacgagatgttcaaccgtgactggagttcagacgtgtgctcttccgatct

SEQ ID NO: 140 - DNA, 66 bp, Artificial Sequence
  Reverse primer
caagcagaagacggcatacgagattggctatcgtgactggagttcagacgtgtgctcttccgatct

SEQ ID NO: 141 - DNA, 66 bp, Artificial Sequence
  Reverse primer
caagcagaagacggcatacgagatctggagtagtgactggagttcagacgtgtgctcttccgatct

SEQ ID NO: 142 - DNA, 66 bp, Artificial Sequence
  Reverse primer
caagcagaagacggcatacgagattctcttccgtgactggagttcagacgtgtgctcttccgatct

SEQ ID NO: 143 - DNA, 66 bp, Artificial Sequence
  Reverse primer
caagcagaagacggcatacgagattctaacgcgtgactggagttcagacgtgtgctcttccgatct

SEQ ID NO: 144 - DNA, 66 bp, Artificial Sequence
  Reverse primer
caagcagaagacggcatacgagatggtcagatgtgactggagttcagacgtgtgctcttccgatct

SEQ ID NO: 145 - DNA, 66 bp, Artificial Sequence
  Reverse primer
caagcagaagacggcatacgagatctctggttgtgactggagttcagacgtgtgctcttccgatct

SEQ ID NO: 146 - DNA, 66 bp, Artificial Sequence
  Reverse primer
caagcagaagacggcatacgagattgtggtacgtgactggagttcagacgtgtgctcttccgatct

SEQ ID NO: 147 - DNA, 66 bp, Artificial Sequence
  Reverse primer
caagcagaagacggcatacgagatcctataccgtgactggagttcagacgtgtgctcttccgatct

SEQ ID NO: 148 - DNA, 66 bp, Artificial Sequence
  Reverse primer
caagcagaagacggcatacgagatttctctcggtgactggagttcagacgtgtgctcttccgatct

SEQ ID NO: 149 - DNA, 66 bp, Artificial Sequence
  Reverse primer
caagcagaagacggcatacgagatgtatgctggtgactggagttcagacgtgtgctcttccgatct

SEQ ID NO: 150 - DNA, 66 bp, Artificial Sequence
  Reverse primer
caagcagaagacggcatacgagataagtcgaggtgactggagttcagacgtgtgctcttccgatct

SEQ ID NO: 151 - DNA, 66 bp, Artificial Sequence
  Reverse primer
caagcagaagacggcatacgagataaccgaaggtgactggagttcagacgtgtgctcttccgatct

SEQ ID NO: 152 - DNA, 66 bp, Artificial Sequence
  Reverse primer
caagcagaagacggcatacgagattgttgtgggtgactggagttcagacgtgtgctcttccgatct

SEQ ID NO: 153 - DNA, 21 bp, Artificial Sequence
  P7 universal primer
caagcagaagacggcatacga

SEQ ID NO: 154 - DNA, 20 bp, Artificial Sequence
  P5 universal primer
aatgatacggcgaccaccga

SEQ ID NO: 155 - DNA, 70 bp, Artificial Sequence
  NEBNext i501 Primer
aatgatacggcgaccaccgagatctacactatagcctacactctttccctacacgacgctcttccgatct

SEQ ID NO: 156 - DNA, 70 bp, Artificial Sequence
  NEBNext i502 Primer
aatgatacggcgaccaccgagatctacacatagaggcacactctttccctacacgacgctcttccgatct

SEQ ID NO: 157 - DNA, 70 bp, Artificial Sequence
  NEBNext i503 Primer
aatgatacggcgaccaccgagatctacaccctatcctacactctttccctacacgacgctcttccgatct

SEQ ID NO: 158 - DNA, 70 bp, Artificial Sequence
  NEBNext i504 Primer
aatgatacggcgaccaccgagatctacacggctctgaacactctttccctacacgacgctcttccgatct

SEQ ID NO: 159 - DNA, 70 bp, Artificial Sequence
  NEBNext i505 Primer
aatgatacggcgaccaccgagatctacacaggcgaagacactctttccctacacgacgctcttccgatct

SEQ ID NO: 160 - DNA, 70 bp, Artificial Sequence
  NEBNext i506 Primer
aatgatacggcgaccaccgagatctacactaatcttaacactctttccctacacgacgctcttccgatct

SEQ ID NO: 161 - DNA, 70 bp, Artificial Sequence
  NEBNext i507 Primer
aatgatacggcgaccaccgagatctacaccaggacgtacactctttccctacacgacgctcttccgatct

SEQ ID NO: 162 - DNA, 70 bp, Artificial Sequence
  NEBNext i508 Primer
aatgatacggcgaccaccgagatctacacgtactgacacactctttccctacacgacgctcttccgatct

SEQ ID NO: 163 - DNA, 100 bp, Artificial Sequence
  UMI14_i701
  misc_feature (65)..(78): n is a, c, g, or t
caagcagaagacggcatacgagatcgtgatgtgactggagttcagacgtgtgctcttccgatctnnnnnnnnnnnnnnaacggacaggatgcagcaaaat

SEQ ID NO: 164 - DNA, 100 bp, Artificial Sequence
  UMI14_i702
  misc_feature (65)..(78): n is a, c, g, or t
caagcagaagacggcatacgagatacatcggtgactggagttcagacgtgtgctcttccgatctnnnnnnnnnnnnnnaacggacaggatgcagcaaaat

SEQ ID NO: 165 - DNA, 100 bp, Artificial Sequence
  UMI14_i703
  misc_feature (65)..(78): n is a, c, g, or t
caagcagaagacggcatacgagatgcctaagtgactggagttcagacgtgtgctcttccgatctnnnnnnnnnnnnnnaacggacaggatgcagcaaaat

SEQ ID NO: 166 - DNA, 100 bp, Artificial Sequence
  UMI14_i704
  misc_feature (65)..(78): n is a, c, g, or t
caagcagaagacggcatacgagattggtcagtgactggagttcagacgtgtgctcttccgatctnnnnnnnnnnnnnnaacggacaggatgcagcaaaat

SEQ ID NO: 167 - DNA, 100 bp, Artificial Sequence
  UMI14_i705
  misc_feature (65)..(78): n is a, c, g, or t
caagcagaagacggcatacgagatcactgtgtgactggagttcagacgtgtgctcttccgatctnnnnnnnnnnnnnnaacggacaggatgcagcaaaat

SEQ ID NO: 168 - DNA, 100 bp, Artificial Sequence
  UMI14_i706
  misc_feature (65)..(78): n is a, c, g, or t
caagcagaagacggcatacgagatattggcgtgactggagttcagacgtgtgctcttccgatctnnnnnnnnnnnnnnaacggacaggatgcagcaaaat

SEQ ID NO: 169 - DNA, 100 bp, Artificial Sequence
  UMI14_i707
  misc_feature (65)..(78): n is a, c, g, or t
caagcagaagacggcatacgagatgatctggtgactggagttcagacgtgtgctcttccgatctnnnnnnnnnnnnnnaacggacaggatgcagcaaaat

SEQ ID NO: 170 - DNA, 100 bp, Artificial Sequence
  UMI14_i708
  misc_feature (65)..(78): n is a, c, g, or t
caagcagaagacggcatacgagattcaagtgtgactggagttcagacgtgtgctcttccgatctnnnnnnnnnnnnnnaacggacaggatgcagcaaaat

SEQ ID NO: 171 - DNA, 100 bp, Artificial Sequence
  UMI14_i709
  misc_feature (65)..(78): n is a, c, g, or t
caagcagaagacggcatacgagatctgatcgtgactggagttcagacgtgtgctcttccgatctnnnnnnnnnnnnnnaacggacaggatgcagcaaaat

SEQ ID NO: 172 - DNA, 100 bp, Artificial Sequence
  UMI14_i710
  misc_feature (65)..(78): n is a, c, g, or t
caagcagaagacggcatacgagataagctagtgactggagttcagacgtgtgctcttccgatctnnnnnnnnnnnnnnaacggacaggatgcagcaaaat

SEQ ID NO: 173 - DNA, 100 bp, Artificial Sequence
  UMI14_i711
  misc_feature (65)..(78): n is a, c, g, or t
caagcagaagacggcatacgagatgtagccgtgactggagttcagacgtgtgctcttccgatctnnnnnnnnnnnnnnaacggacaggatgcagcaaaat

SEQ ID NO: 174 - DNA, 100 bp, Artificial Sequence
  UMI14_i712
  misc_feature (65)..(78): n is a, c, g, or t
caagcagaagacggcatacgagattacaaggtgactggagttcagacgtgtgctcttccgatctnnnnnnnnnnnnnnaacggacaggatgcagcaaaat